European Patent Specification EP 3 677 678 B1, published January 31, 2024. Title: MAKING AND USING IN VITRO-SYNTHESIZED ssRNA FOR INTRODUCING INTO MAMMALIAN CELLS TO INDUCE A BIOLOGICAL OR BIOCHEMICAL EFFECT. Applicant: CELLSCRIPT, LLC. Application EP. The sequence listing filed with the application follows.

SEQUENCE LISTING (16 sequences)

SEQ ID NO: 1 - DNA, 269 bp, Artificial sequence
  Synthetic
taatacgactcactatagggtaatacaagcttgcttgttctttttgcagaagctcagaataaacgctcaactttggcagatctgatatcactagtgactgactaggatctggttaccactaaaccagcctcaagaacacccgaatggagtctctaagctacataataccaacttacacttacaaaatgttgtcccccaaaatgtagccattcgtatctgctcctaataaaaagaaagtttcttcacattctggatcctctagagtcgac

SEQ ID NO: 2 - DNA, 4017 bp, Artificial sequence
  Synthetic
tcgcgcgtttcggtgatgacggtgaaaacctctgacacatgcagctcccggagacggtcacagcttgtctgtaagcggatgccgggagcagacaagcccgtcagggcgcgtcagcgggtgttggcgggtgtcggggctggcttaactatgcggcatcagagcagattgtactgagagtgcaccatatgcggtgtgaaataccgcacagatgcgtaaggagaaaataccgcatcaggcgccattcgccattcaggctgcgcaactgttgggaagggcgatcggtgcgggcctcttcgctattacgccagctggcgaaagggggatgtgctgcaaggcgattaagttgggtaacgccagggttttcccagtcacgacgttgtaaaacgacggccagtgaattctaatacgactcactatagggtaatacaagcttgcttgttctttttgcagaagctcagaataaacgctcaactttggcagatctcggtcgccaccatggcgggacacctggcttcagattttgccttctcgccccctccaggtggtggaggtgatgggccaggggggccggagccgggctgggttgatcctcggacctggctaagcttccaaggccctcctggagggccaggaatcgggccgggggttgggccaggctctgaggtgtgggggattcccccatgccccccgccgtatgagttctgtggggggatggcgtactgtgggccccaggttggagtggggctagtgccccaaggcggcttggagacctctcagcctgagggcgaagcaggagtcggggtggagagcaactccgatggggcctccccggagccctgcaccgtcacccctggtgccgtgaagctggagaaggagaagctggagcaaaacccggaggagtcccaggacatcaaagctctgcagaaagaactcgagcaatttgccaagctcctgaagcagaagaggatcaccctgggatatacacaggccgatgtggggctcaccctgggggttctatttgggaaggtattcagccaaacgaccatctgccgctttgaggctctgcagcttagcttcaagaacatgtgtaagctgcggcccttgctgcagaagtgggtggaggaagctgacaacaatgaaaatcttcaggagatatgcaaagcagaaaccctcgtgcaggcccgaaagagaaagcgaaccagtatcgagaaccgagtgagaggcaacctggagaatttgttcctgcagtgcccgaaacccacactgcagcagatcagccacatcgcccagcagcttgggctcgagaaggatgtggtccgagtgtggttctgtaaccggcgccagaagggcaagcgatcaagcagcgactatgcacaacgagaggattttgaggctgctgggtctcctttctcagggggaccagtgtcctttcctctggccccagggccccattttggtaccccaggctatgggagccctcacttcactgcactgtactcctcggtccctttccctgagggggaagcctttccccctgtctctgtcaccactctgggctctcccatgcattcaaactgagatatcactagtgactgactaggatctggttaccactaaaccagcctcaagaacacccgaatggagtctctaagctacataataccaacttacactttacaaaatgttgtcccccaaaatgtagccattcgtatctgctcctaataaaaagaaagtttcttcacattctggatcctctagagtcgacctgcaggcatgcaagcttggcgtaatcatggtcatagctgtttcctgtgtgaaattgttatccgctcacaattccacacaacatacgagccggaagcataaagtgtaaagcctggggtgcctaatgagtgagctaactcacattaattgcgttgcgctcactgcccgctttccagtcgggaaacctgtcgtgccagctgcattaatgaatcggccaacgcgcggggagaggcggtttgcgtattgggcgctcttccgcttcctcgctcactgactcgctgcgctcggtcgttcggctgcggcgagcggtatcagctcactcaaaggcggtaatacggttatccacagaatcaggggataacgcaggaaagaacatgtgagcaaaaggccagcaaaaggccaggaaccgtaaaaaggccgcgttgctggcgtttttccataggctccgcccccctgacgagcatcacaaaaatcgacgctcaagtcagaggtggcgaaacccgacaggactataaagataccaggcgtttccccctggaagctccctcgtgcgctctcctgttccgaccctgccgcttaccggatacctgtccgcctttctcccttcgggaagcgtggcgctttctcatagctcacgctgtaggtatctcagttcggtgtaggtcgttcgctccaagctgggctgtgtgcacgaaccccccgttcagcccgaccgctgcgccttatccggtaactatcgtcttgagtccaacccggtaagacacgacttatcgccactggcagcagccactggtaacaggattagcagagcgaggtatgtaggcggtgctacagagttcttgaagtggtggcctaactacggctacactagaagaacagtatttggtatctgcgctctgctgaagccagttaccttcggaaaaagagttggtagctcttgatccggcaaacaaaccaccgctggtagcggtggtttttttgtttgcaagcagcagattacgcgcagaaaaaaaggatctcaagaagatcctttgatcttttctacggggtctgacgctcagtggaacgaaaactcacgttaagggattttggtcatgagattatcaaaaaggatcttcacctagatccttttaaattaaaaatgaagttttaaatcaatctaaagtatatatgagtaaacttggtctgacagttaccaatgcttaatcagtgaggcacctatctcagcgatctgtctatttcgttcatccatagttgcctgactccccgtcgtgtagataactacgatacgggagggcttaccatctggccccagtgctgcaatgataccgcgagacccacgctcaccggctccagatttatcagcaataaaccagccagccggaagggccgagcgcagaagtggtcctgcaactttatccgcctccatccagtctattaattgttgccgggaagctagagtaagtagttcgccagttaatagtttgcgcaacgttgttgccattgctacaggcatcgtggtgtcacgctcgtcgtttggtatggcttcattcagctccggttcccaacgatcaaggcgagttacatgatcccccatgttgtgcaaaaaagcggttagctccttcggtcctccgatcgttgtcagaagtaagttggccgcagtgttatcactcatggttatggcagcactgcataattctcttactgtcatgccatccgtaagatgcttttctgtgactggtgagtactcaaccaagtcattctgagaatagtgtatgcggcgaccgagttgctcttgcccggcgtcaatacgggataataccgcgccacatagcagaactttaaaagtgctcatcattggaaaacgttcttcggggcgaaaactctcaaggatcttaccgctgttgagatccagttcgatgtaacccactcgtgcacccaactgatcttcagcatcttttactttcaccagcgtttctgggtgagcaaaaacaggaaggcaaaatgccgcaaaaaagggaataagggcgacacggaaatgttgaatactcatactcttcctttttcaatattattgaagcatttatcagggttattgtctcatgagcggatacatatttgaatgtatttagaaaaataaacaaataggggttccgcgcacatttccccgaaaagtgccacctgacgtctaagaaaccattattatcatgacattaacctataaaaataggcgtatcacgaggccctttcgtc

SEQ ID NO: 3 - DNA, 3888 bp, Artificial sequence
  Synthetic
tcgcgcgtttcggtgatgacggtgaaaacctctgacacatgcagctcccggagacggtcacagcttgtctgtaagcggatgccgggagcagacaagcccgtcagggcgcgtcagcgggtgttggcgggtgtcggggctggcttaactatgcggcatcagagcagattgtactgagagtgcaccatatgcggtgtgaaataccgcacagatgcgtaaggagaaaataccgcatcaggcgccattcgccattcaggctgcgcaactgttgggaagggcgatcggtgcgggcctcttcgctattacgccagctggcgaaagggggatgtgctgcaaggcgattaagttgggtaacgccagggttttcccagtcacgacgttgtaaaacgacggccagtgaattctaatacgactcactatagggtaatacaagcttgcttgttctttttgcagaagctcagaataaacgctcaactttggcagatctcggtcgccaccatgtacaacatgatggagacggagctgaagccgccgggcccgcagcaaacttcggggggcggcggcggcaactccaccgcggcggcggccggcggcaaccagaaaaacagcccggaccgcgtcaagcggcccatgaatgccttcatggtgtggtcccgcgggcagcggcgcaagatggcccaggagaaccccaagatgcacaactcggagatcagcaagcgcctgggcgccgagtggaaacttttgtcggagacggagaagcggccgttcatcgacgaggctaagcggctgcgagcgctgcacatgaaggagcacccggattataaataccggccccggcggaaaaccaagacgctcatgaagaaggataagtacacgctgcccggcgggctgctggcccccggcggcaatagcatggcgagcggggtcggggtgggcgccggcctgggcgcgggcgtgaaccagcgcatggacagttacgcgcacatgaacggctggagcaacggcagctacagcatgatgcaggaccagctgggctacccgcagcacccgggcctcaatgcgcacggcgcagcgcagatgcagcccatgcaccgctacgacgtgagcgccctgcagtacaactccatgaccagctcgcagacctacatgaacggctcgcccacctacagcatgtcctactcgcagcagggcacccctggcatggctcttggctccatgggttcggtggtcaagtccgaggccagctccagcccccctgtggttacctcttcctcccactccagggcgccctgccaggccggggacctccgggacatgatcagcatgtatctccccggcgccgaggtgccggaacccgccgcccccagcagacttcacatgtcccagcactaccagagcggcccggtgcccggcacggccattaacggcacactgcccctctcacacatgtgagatatcactagtgactgactaggatctggttaccactaaaccagcctcaagaacacccgaatggagtctctaagctacataataccaacttacactttacaaaatgttgtcccccaaaatgtagccattcgtatctgctcctaataaaaagaaagtttcttcacattctggatcctctagagtcgacctgcaggcatgcaagcttggcgtaatcatggtcatagctgtttcctgtgtgaaattgttatccgctcacaattccacacaacatacgagccggaagcataaagtgtaaagcctggggtgcctaatgagtgagctaactcacattaattgcgttgcgctcactgcccgctttccagtcgggaaacctgtcgtgccagctgcattaatgaatcggccaacgcgcggggagaggcggtttgcgtattgggcgctcttccgcttcctcgctcactgactcgctgcgctcggtcgttcggctgcggcgagcggtatcagctcactcaaaggcggtaatacggttatccacagaatcaggggataacgcaggaaagaacatgtgagcaaaaggccagcaaaaggccaggaaccgtaaaaaggccgcgttgctggcgtttttccataggctccgcccccctgacgagcatcacaaaaatcgacgctcaagtcagaggtggcgaaacccgacaggactataaagataccaggcgtttccccctggaagctccctcgtgcgctctcctgttccgaccctgccgcttaccggatacctgtccgcctttctcccttcgggaagcgtggcgctttctcatagctcacgctgtaggtatctcagttcggtgtaggtcgttcgctccaagctgggctgtgtgcacgaaccccccgttcagcccgaccgctgcgccttatccggtaactatcgtcttgagtccaacccggtaagacacgacttatcgccactggcagcagccactggtaacaggattagcagagcgaggtatgtaggcggtgctacagagttcttgaagtggtggcctaactacggctacactagaagaacagtatttggtatctgcgctctgctgaagccagttaccttcggaaaaagagttggtagctcttgatccggcaaacaaaccaccgctggtagcggtggtttttttgtttgcaagcagcagattacgcgcagaaaaaaaggatctcaagaagatcctttgatcttttctacggggtctgacgctcagtggaacgaaaactcacgttaagggattttggtcatgagattatcaaaaaggatcttcacctagatccttttaaattaaaaatgaagttttaaatcaatctaaagtatatatgagtaaacttggtctgacagttaccaatgcttaatcagtgaggcacctatctcagcgatctgtctatttcgttcatccatagttgcctgactccccgtcgtgtagataactacgatacgggagggcttaccatctggccccagtgctgcaatgataccgcgagacccacgctcaccggctccagatttatcagcaataaaccagccagccggaagggccgagcgcagaagtggtcctgcaactttatccgcctccatccagtctattaattgttgccgggaagctagagtaagtagttcgccagttaatagtttgcgcaacgttgttgccattgctacaggcatcgtggtgtcacgctcgtcgtttggtatggcttcattcagctccggttcccaacgatcaaggcgagttacatgatcccccatgttgtgcaaaaaagcggttagctccttcggtcctccgatcgttgtcagaagtaagttggccgcagtgttatcactcatggttatggcagcactgcataattctcttactgtcatgccatccgtaagatgcttttctgtgactggtgagtactcaaccaagtcattctgagaatagtgtatgcggcgaccgagttgctcttgcccggcgtcaatacgggataataccgcgccacatagcagaactttaaaagtgctcatcattggaaaacgttcttcggggcgaaaactctcaaggatcttaccgctgttgagatccagttcgatgtaacccactcgtgcacccaactgatcttcagcatcttttactttcaccagcgtttctgggtgagcaaaaacaggaaggcaaaatgccgcaaaaaagggaataagggcgacacggaaatgttgaatactcatactcttcctttttcaatattattgaagcatttatcagggttattgtctcatgagcggatacatatttgaatgtatttagaaaaataaacaaataggggttccgcgcacatttccccgaaaagtgccacctgacgtctaagaaaccattattatcatgacattaacctataaaaataggcgtatcacgaggccctttcgtc

SEQ ID NO: 4 - DNA, 4369 bp, Artificial sequence
  Synthetic
tcgcgcgtttcggtgatgacggtgaaaacctctgacacatgcagctcccggagacggtcacagcttgtctgtaagcggatgccgggagcagacaagcccgtcagggcgcgtcagcgggtgttggcgggtgtcggggctggcttaactatgcggcatcagagcagattgtactgagagtgcaccatatgcggtgtgaaataccgcacagatgcgtaaggagaaaataccgcatcaggcgccattcgccattcaggctgcgcaactgttgggaagggcgatcggtgcgggcctcttcgctattacgccagctggcgaaagggggatgtgctgcaaggcgattaagttgggtaacgccagggttttcccagtcacgacgttgtaaaacgacggccagtgaattctaatacgactcactatagggtaatacaagcttgcttgttctttttgcagaagctcagaataaacgctcaactttggcagatctgccaccatgaggcagccacctggcgagtctgacatggctgtcagcgacgcgctgctcccatctttctccacgttcgcgtctggcccggcgggaagggagaagacactgcgtcaagcaggtgccccgaataaccgctggcgggaggagctctcccacatgaagcgacttcccccagtgcttcccggccgcccctatgacctggcggcggcgaccgtggccacagacctggagagcggcggagccggtgcggcttgcggcggtagcaacctggcgcccctacctcggagagagaccgaggagttcaacgatctcctggacctggactttattctctccaattcgctgacccatcctccggagtcagtggccgccaccgtgtcctcgtcagcgtcagcctcctcttcgtcgtcgccgtcgagcagcggccctgccagcgcgccctccacctgcagcttcacctatccgatccgggccgggaacgacccgggcgtggcgccgggcggcacgggcggaggcctcctctatggcagggagtccgctccccctccgacggctcccttcaacctggcggacatcaacgacgtgagcccctcgggcggcttcgtggccgagctcctgcggccagaattggacccggtgtacattccgccgcagcagccgcagccgccaggtggcgggctgatgggcaagttcgtgctgaaggcgtcgctgagcgcccctggcagcgagtacggcagcccgtcggtcatcagcgtcagcaaaggcagccctgacggcagccacccggtggtggtggcgccctacaacggcgggccgccgcgcacgtgccccaagatcaagcaggaggcggtctcttcgtgcacccacttgggcgctggaccccctctcagcaatggccaccggccggctgcacacgacttccccctggggcggcagctccccagcaggactaccccgaccctgggtcttgaggaagtgctgagcagcagggactgtcaccctgccctgccgcttcctcccggcttccatccccacccggggcccaattacccatccttcctgcccgatcagatgcagccgcaagtcccgccgctccattaccaagagctcatgccacccggttcctgcatgccagaggagcccaagccaaagaggggaagacgatcgtggccccggaaaaggaccgccacccacacttgtgattacgcgggctgcggcaaaacctacacaaagagttcccatctcaaggcacacctgcgaacccacacaggtgagaaaccttaccactgtgactgggacggctgtggatggaaattcgcccgctcagatgaactgaccaggcactaccgtaaacacacggggcaccgcccgttccagtgccaaaaatgcgaccgagcattttccaggtcggaccacctcgccttacacatgaagaggcatttttaagatatcactagtgactgactaggatctggttaccactaaaccagcctcaagaacacccgaatggagtctctaagctacataataccaacttacactttacaaaatgttgtcccccaaaatgtagccattcgtatctgctcctaataaaaagaaagtttcttcacattctggatcctctagagtcgacctgcaggcatgcaagcttggcgtaatcatggtcatagctgtttcctgtgtgaaattgttatccgctcacaattccacacaacatacgagccggaagcataaagtgtaaagcctggggtgcctaatgagtgagctaactcacattaattgcgttgcgctcactgcccgctttccagtcgggaaacctgtcgtgccagctgcattaatgaatcggccaacgcgcggggagaggcggtttgcgtattgggcgctcttccgcttcctcgctcactgactcgctgcgctcggtcgttcggctgcggcgagcggtatcagctcactcaaaggcggtaatacggttatccacagaatcaggggataacgcaggaaagaacatgtgagcaaaaggccagcaaaaggccaggaaccgtaaaaaggccgcgttgctggcgtttttccataggctccgcccccctgacgagcatcacaaaaatcgacgctcaagtcagaggtggcgaaacccgacaggactataaagataccaggcgtttccccctggaagctccctcgtgcgctctcctgttccgaccctgccgcttaccggatacctgtccgcctttctcccttcgggaagcgtggcgctttctcatagctcacgctgtaggtatctcagttcggtgtaggtcgttcgctccaagctgggctgtgtgcacgaaccccccgttcagcccgaccgctgcgccttatccggtaactatcgtcttgagtccaacccggtaagacacgacttatcgccactggcagcagccactggtaacaggattagcagagcgaggtatgtaggcggtgctacagagttcttgaagtggtggcctaactacggctacactagaagaacagtatttggtatctgcgctctgctgaagccagttaccttcggaaaaagagttggtagctcttgatccggcaaacaaaccaccgctggtagcggtggtttttttgtttgcaagcagcagattacgcgcagaaaaaaaggatctcaagaagatcctttgatcttttctacggggtctgacgctcagtggaacgaaaactcacgttaagggattttggtcatgagattatcaaaaaggatcttcacctagatccttttaaattaaaaatgaagttttaaatcaatctaaagtatatatgagtaaacttggtctgacagttaccaatgcttaatcagtgaggcacctatctcagcgatctgtctatttcgttcatccatagttgcctgactccccgtcgtgtagataactacgatacgggagggcttaccatctggccccagtgctgcaatgataccgcgagacccacgctcaccggctccagatttatcagcaataaaccagccagccggaagggccgagcgcagaagtggtcctgcaactttatccgcctccatccagtctattaattgttgccgggaagctagagtaagtagttcgccagttaatagtttgcgcaacgttgttgccattgctacaggcatcgtggtgtcacgctcgtcgtttggtatggcttcattcagctccggttcccaacgatcaaggcgagttacatgatcccccatgttgtgcaaaaaagcggttagctccttcggtcctccgatcgttgtcagaagtaagttggccgcagtgttatcactcatggttatggcagcactgcataattctcttactgtcatgccatccgtaagatgcttttctgtgactggtgagtactcaaccaagtcattctgagaatagtgtatgcggcgaccgagttgctcttgcccggcgtcaatacgggataataccgcgccacatagcagaactttaaaagtgctcatcattggaaaacgttcttcggggcgaaaactctcaaggatcttaccgctgttgagatccagttcgatgtaacccactcgtgcacccaactgatcttcagcatcttttactttcaccagcgtttctgggtgagcaaaaacaggaaggcaaaatgccgcaaaaaagggaataagggcgacacggaaatgttgaatactcatactcttcctttttcaatattattgaagcatttatcagggttattgtctcatgagcggatacatatttgaatgtatttagaaaaataaacaaataggggttccgcgcacatttccccgaaaagtgccacctgacgtctaagaaaccattattatcatgacattaacctataaaaataggcgtatcacgaggccctttcgtc

SEQ ID NO: 5 - DNA, 3559 bp, Artificial sequence
  Synthetic
tcgcgcgtttcggtgatgacggtgaaaacctctgacacatgcagctcccggagacggtcacagcttgtctgtaagcggatgccgggagcagacaagcccgtcagggcgcgtcagcgggtgttggcgggtgtcggggctggcttaactatgcggcatcagagcagattgtactgagagtgcaccatatgcggtgtgaaataccgcacagatgcgtaaggagaaaataccgcatcaggcgccattcgccattcaggctgcgcaactgttgggaagggcgatcggtgcgggcctcttcgctattacgccagctggcgaaagggggatgtgctgcaaggcgattaagttgggtaacgccagggttttcccagtcacgacgttgtaaaacgacggccagtgaattctaatacgactcactatagggtaatacaagcttgcttgttctttttgcagaagctcagaataaacgctcaactttggcagatctgccaccatgggctccgtgtccaaccagcagtttgcaggtggctgcgccaaggcggcagaagaggcgcccgaggaggcgccggaggacgcggcccgggcggcggacgagcctcagctgctgcacggtgcgggcatctgtaagtggttcaacgtgcgcatggggttcggcttcctgtccatgaccgcccgcgccggggtcgcgctcgaccccccagtggatgtctttgtgcaccagagtaagctgcacatggaagggttccggagcttgaaggagggtgaggcagtggagttcacctttaagaagtcagccaagggtctggaatccatccgtgtcaccggacctggtggagtattctgtattgggagtgagaggcggccaaaaggaaagagcatgcagaagcgcagatcaaaaggagacaggtgctacaactgtggaggtctagatcatcatgccaaggaatgcaagctgccaccccagcccaagaagtgccacttctgccagagcatcagccatatggtagcctcatgtccgctgaaggcccagcagggccctagtgcacagggaaagccaacctactttcgagaggaagaagaagaaatccacagccctaccctgctcccggaggcacagaattgagatatcactagtgactgactaggatctggttaccactaaaccagcctcaagaacacccgaatggagtctctaagctacataataccaacttacactttacaaaatgttgtcccccaaaatgtagccattcgtatctgctcctaataaaaagaaagtttcttcacattctggatcctctagagtcgacctgcaggcatgcaagcttggcgtaatcatggtcatagctgtttcctgtgtgaaattgttatccgctcacaattccacacaacatacgagccggaagcataaagtgtaaagcctggggtgcctaatgagtgagctaactcacattaattgcgttgcgctcactgcccgctttccagtcgggaaacctgtcgtgccagctgcattaatgaatcggccaacgcgcggggagaggcggtttgcgtattgggcgctcttccgcttcctcgctcactgactcgctgcgctcggtcgttcggctgcggcgagcggtatcagctcactcaaaggcggtaatacggttatccacagaatcaggggataacgcaggaaagaacatgtgagcaaaaggccagcaaaaggccaggaaccgtaaaaaggccgcgttgctggcgtttttccataggctccgcccccctgacgagcatcacaaaaatcgacgctcaagtcagaggtggcgaaacccgacaggactataaagataccaggcgtttccccctggaagctccctcgtgcgctctcctgttccgaccctgccgcttaccggatacctgtccgcctttctcccttcgggaagcgtggcgctttctcatagctcacgctgtaggtatctcagttcggtgtaggtcgttcgctccaagctgggctgtgtgcacgaaccccccgttcagcccgaccgctgcgccttatccggtaactatcgtcttgagtccaacccggtaagacacgacttatcgccactggcagcagccactggtaacaggattagcagagcgaggtatgtaggcggtgctacagagttcttgaagtggtggcctaactacggctacactagaagaacagtatttggtatctgcgctctgctgaagccagttaccttcggaaaaagagttggtagctcttgatccggcaaacaaaccaccgctggtagcggtggtttttttgtttgcaagcagcagattacgcgcagaaaaaaaggatctcaagaagatcctttgatcttttctacggggtctgacgctcagtggaacgaaaactcacgttaagggattttggtcatgagattatcaaaaaggatcttcacctagatccttttaaattaaaaatgaagttttaaatcaatctaaagtatatatgagtaaacttggtctgacagttaccaatgcttaatcagtgaggcacctatctcagcgatctgtctatttcgttcatccatagttgcctgactccccgtcgtgtagataactacgatacgggagggcttaccatctggccccagtgctgcaatgataccgcgagacccacgctcaccggctccagatttatcagcaataaaccagccagccggaagggccgagcgcagaagtggtcctgcaactttatccgcctccatccagtctattaattgttgccgggaagctagagtaagtagttcgccagttaatagtttgcgcaacgttgttgccattgctacaggcatcgtggtgtcacgctcgtcgtttggtatggcttcattcagctccggttcccaacgatcaaggcgagttacatgatcccccatgttgtgcaaaaaagcggttagctccttcggtcctccgatcgttgtcagaagtaagttggccgcagtgttatcactcatggttatggcagcactgcataattctcttactgtcatgccatccgtaagatgcttttctgtgactggtgagtactcaaccaagtcattctgagaatagtgtatgcggcgaccgagttgctcttgcccggcgtcaatacgggataataccgcgccacatagcagaactttaaaagtgctcatcattggaaaacgttcttcggggcgaaaactctcaaggatcttaccgctgttgagatccagttcgatgtaacccactcgtgcacccaactgatcttcagcatcttttactttcaccagcgtttctgggtgagcaaaaacaggaaggcaaaatgccgcaaaaaagggaataagggcgacacggaaatgttgaatactcatactcttcctttttcaatattattgaagcatttatcagggttattgtctcatgagcggatacatatttgaatgtatttagaaaaataaacaaataggggttccgcgcacatttccccgaaaagtgccacctgacgtctaagaaaccattattatcatgacattaacctataaaaataggcgtatcacgaggccctttcgtc

SEQ ID NO: 6 - DNA, 3847 bp, Artificial sequence
  Synthetic
tcgcgcgtttcggtgatgacggtgaaaacctctgacacatgcagctcccggagacggtcacagcttgtctgtaagcggatgccgggagcagacaagcccgtcagggcgcgtcagcgggtgttggcgggtgtcggggctggcttaactatgcggcatcagagcagattgtactgagagtgcaccatatgcggtgtgaaataccgcacagatgcgtaaggagaaaataccgcatcaggcgccattcgccattcaggctgcgcaactgttgggaagggcgatcggtgcgggcctcttcgctattacgccagctggcgaaagggggatgtgctgcaaggcgattaagttgggtaacgccagggttttcccagtcacgacgttgtaaaacgacggccagtgaattctaatacgactcactatagggtaatacaagcttgcttgttctttttgcagaagctcagaataaacgctcaactttggcagatctgccaccatgagtgtggatccagcttgtccccaaagcttgccttgctttgaagcatccgactgtaaagaatcttcacctatgcctgtgatttgtgggcctgaagaaaactatccatccttgcaaatgtcttctgctgagatgcctcacacagagactgtctctcctcttccttcctccatggatctgcttattcaggacagccctgattcttccaccagtcccaaaggcaaacaacccacttctgcagagaatagtgtcgcaaaaaaggaagacaaggtcccggtcaagaaacagaagaccagaactgtgttctcttccacccagctgtgtgtactcaatgatagatttcagagacagaaatacctcagcctccagcagatgcaagaactctccaacatcctgaacctcagctacaaacaggtgaagacctggttccagaaccagagaatgaaatctaagaggtggcagaaaaacaactggccgaagaatagcaatggtgtgacgcagaaggcctcagcacctacctaccccagcctctactcttcctaccaccagggatgcctggtgaacccgactgggaaccttccaatgtggagcaaccagacctggaacaattcaacctggagcaaccagacccagaacatccagtcctggagcaaccactcctggaacactcagacctggtgcacccaatcctggaacaatcaggcctggaacagtcccttctataactgtggagaggaatctctgcagtcctgcatgcacttccagccaaattctcctgccagtgacttggaggctgccttggaagctgctggggaaggccttaatgtaatacagcagaccactaggtattttagtactccacaaaccatggatttattcctaaactactccatgaacatgcaacctgaagacgtgtgagatatcactagtgactgactaggatctggttaccactaaaccagcctcaagaacacccgaatggagtctctaagctacataataccaacttacactttacaaaatgttgtcccccaaaatgtagccattcgtatctgctcctaataaaaagaaagtttcttcacattctggatcctctagagtcgacctgcaggcatgcaagcttggcgtaatcatggtcatagctgtttcctgtgtgaaattgttatccgctcacaattccacacaacatacgagccggaagcataaagtgtaaagcctggggtgcctaatgagtgagctaactcacattaattgcgttgcgctcactgcccgctttccagtcgggaaacctgtcgtgccagctgcattaatgaatcggccaacgcgcggggagaggcggtttgcgtattgggcgctcttccgcttcctcgctcactgactcgctgcgctcggtcgttcggctgcggcgagcggtatcagctcactcaaaggcggtaatacggttatccacagaatcaggggataacgcaggaaagaacatgtgagcaaaaggccagcaaaaggccaggaaccgtaaaaaggccgcgttgctggcgtttttccataggctccgcccccctgacgagcatcacaaaaatcgacgctcaagtcagaggtggcgaaacccgacaggactataaagataccaggcgtttccccctggaagctccctcgtgcgctctcctgttccgaccctgccgcttaccggatacctgtccgcctttctcccttcgggaagcgtggcgctttctcatagctcacgctgtaggtatctcagttcggtgtaggtcgttcgctccaagctgggctgtgtgcacgaaccccccgttcagcccgaccgctgcgccttatccggtaactatcgtcttgagtccaacccggtaagacacgacttatcgccactggcagcagccactggtaacaggattagcagagcgaggtatgtaggcggtgctacagagttcttgaagtggtggcctaactacggctacactagaagaacagtatttggtatctgcgctctgctgaagccagttaccttcggaaaaagagttggtagctcttgatccggcaaacaaaccaccgctggtagcggtggtttttttgtttgcaagcagcagattacgcgcagaaaaaaaggatctcaagaagatcctttgatcttttctacggggtctgacgctcagtggaacgaaaactcacgttaagggattttggtcatgagattatcaaaaaggatcttcacctagatccttttaaattaaaaatgaagttttaaatcaatctaaagtatatatgagtaaacttggtctgacagttaccaatgcttaatcagtgaggcacctatctcagcgatctgtctatttcgttcatccatagttgcctgactccccgtcgtgtagataactacgatacgggagggcttaccatctggccccagtgctgcaatgataccgcgagacccacgctcaccggctccagatttatcagcaataaaccagccagccggaagggccgagcgcagaagtggtcctgcaactttatccgcctccatccagtctattaattgttgccgggaagctagagtaagtagttcgccagttaatagtttgcgcaacgttgttgccattgctacaggcatcgtggtgtcacgctcgtcgtttggtatggcttcattcagctccggttcccaacgatcaaggcgagttacatgatcccccatgttgtgcaaaaaagcggttagctccttcggtcctccgatcgttgtcagaagtaagttggccgcagtgttatcactcatggttatggcagcactgcataattctcttactgtcatgccatccgtaagatgcttttctgtgactggtgagtactcaaccaagtcattctgagaatagtgtatgcggcgaccgagttgctcttgcccggcgtcaatacgggataataccgcgccacatagcagaactttaaaagtgctcatcattggaaaacgttcttcggggcgaaaactctcaaggatcttaccgctgttgagatccagttcgatgtaacccactcgtgcacccaactgatcttcagcatcttttactttcaccagcgtttctgggtgagcaaaaacaggaaggcaaaatgccgcaaaaaagggaataagggcgacacggaaatgttgaatactcatactcttcctttttcaatattattgaagcatttatcagggttattgtctcatgagcggatacatatttgaatgtatttagaaaaataaacaaataggggttccgcgcacatttccccgaaaagtgccacctgacgtctaagaaaccattattatcatgacattaacctataaaaataggcgtatcacgaggccctttcgtc

SEQ ID NO: 7 - DNA, 4304 bp, Artificial sequence
  Synthetic
tcgcgcgtttcggtgatgacggtgaaaacctctgacacatgcagctcccggagacggtcacagcttgtctgtaagcggatgccgggagcagacaagcccgtcagggcgcgtcagcgggtgttggcgggtgtcggggctggcttaactatgcggcatcagagcagattgtactgagagtgcaccatatgcggtgtgaaataccgcacagatgcgtaaggagaaaataccgcatcaggcgccattcgccattcaggctgcgcaactgttgggaagggcgatcggtgcgggcctcttcgctattacgccagctggcgaaagggggatgtgctgcaaggcgattaagttgggtaacgccagggttttcccagtcacgacgttgtaaaacgacggccagtgaattctaatacgactcactatagggtaatacaagcttgcttgttctttttgcagaagctcagaataaacgctcaactttggcagatctgataattcgccaccatggatttttttcgggtagtggaaaaccagcagcctcccgcgacgatgcccctcaacgttagcttcaccaacaggaactatgacctcgactacgactcggtgcagccgtatttctactgcgacgaggaggagaacttctaccagcagcagcagcagagcgagctgcagcccccggcgcccagcgaggatatctggaagaaattcgagctgctgcccaccccgcccctgtcccctagccgccgctccgggctctgctcgccctcctacgttgcggtcacacccttctcccttcggggagacaacgacggcggtggcgggagcttctccacggccgaccagctggagatggtgaccgagctgctgggaggagacatggtgaaccagagtttcatctgcgacccggacgacgagaccttcatcaaaaacatcatcatccaggactgtatgtggagcggcttctcggccgccgccaagctcgtctcagagaagctggcctcctaccaggctgcgcgcaaagacagcggcagcccgaaccccgcccgcggccacagcgtctgctccacctccagcttgtacctgcaggatctgagcgccgccgcctcagagtgcatcgacccctcggtggtcttcccctaccctctcaacgacagcagctcgcccaagtcctgcgcctcgcaagactccagcgccttctctccgtcctcggattctctgctctcctcgacggagtcctccccgcagggcagccccgagcccctggtgctccatgaggagacaccgcccaccaccagcagcgactctgaggaggaacaagaagatgaggaagaaatcgatgttgtttctgtggaaaagaggcaggctcctggcaaaaggtcagagtctggatcaccttctgctggaggccacagcaaacctcctcacagcccactggtcctcaagaggtgccacgtctccacacatcagcacaactacgcagcgcctccctccactcggaaggactatcctgctgccaagagggtcaagttggacagtgtcagagtcctgagacagatcagcaacaaccgaaaatgcaccagccccaggtcctcggacaccgaggagaatgtcaagaggcgaacacacaacgtcttggagcgccagaggaggaacgagctaaaacggagcttttttgccctgcgtgaccagatcccggagttggaaaacaatgaaaaggcccccaaggtagttatccttaaaaaagccacagcatacatcctgtccgtccaagcagaggagcaaaagctcatttctgaagaggacttgttgcggaaacgacgagaacagttgaaacacaaacttgaacagctacggaactcttgtgcgtaaggatcatcactagtgactgactaggatctggttaccactaaaccagcctcaagaacacccgaatggagtctctaagctacataataccaacttacactttacaaaatgttgtcccccaaaatgtagccattcgtatctgctcctaataaaaagaaagtttcttcacattctggatcctctagagtcgacctgcaggcatgcaagcttggcgtaatcatggtcatagctgtttcctgtgtgaaattgttatccgctcacaattccacacaacatacgagccggaagcataaagtgtaaagcctggggtgcctaatgagtgagctaactcacattaattgcgttgcgctcactgcccgctttccagtcgggaaacctgtcgtgccagctgcattaatgaatcggccaacgcgcggggagaggcggtttgcgtattgggcgctcttccgcttcctcgctcactgactcgctgcgctcggtcgttcggctgcggcgagcggtatcagctcactcaaaggcggtaatacggttatccacagaatcaggggataacgcaggaaagaacatgtgagcaaaaggccagcaaaaggccaggaaccgtaaaaaggccgcgttgctggcgtttttccataggctccgcccccctgacgagcatcacaaaaatcgacgctcaagtcagaggtggcgaaacccgacaggactataaagataccaggcgtttccccctggaagctccctcgtgcgctctcctgttccgaccctgccgcttaccggatacctgtccgcctttctcccttcgggaagcgtggcgctttctcatagctcacgctgtaggtatctcagttcggtgtaggtcgttcgctccaagctgggctgtgtgcacgaaccccccgttcagcccgaccgctgcgccttatccggtaactatcgtcttgagtccaacccggtaagacacgacttatcgccactggcagcagccactggtaacaggattagcagagcgaggtatgtaggcggtgctacagagttcttgaagtggtggcctaactacggctacactagaagaacagtatttggtatctgcgctctgctgaagccagttaccttcggaaaaagagttggtagctcttgatccggcaaacaaaccaccgctggtagcggtggtttttttgtttgcaagcagcagattacgcgcagaaaaaaaggatctcaagaagatcctttgatcttttctacggggtctgacgctcagtggaacgaaaactcacgttaagggattttggtcatgagattatcaaaaaggatcttcacctagatccttttaaattaaaaatgaagttttaaatcaatctaaagtatatatgagtaaacttggtctgacagttaccaatgcttaatcagtgaggcacctatctcagcgatctgtctatttcgttcatccatagttgcctgactccccgtcgtgtagataactacgatacgggagggcttaccatctggccccagtgctgcaatgataccgcgagacccacgctcaccggctccagatttatcagcaataaaccagccagccggaagggccgagcgcagaagtggtcctgcaactttatccgcctccatccagtctattaattgttgccgggaagctagagtaagtagttcgccagttaatagtttgcgcaacgttgttgccattgctacaggcatcgtggtgtcacgctcgtcgtttggtatggcttcattcagctccggttcccaacgatcaaggcgagttacatgatcccccatgttgtgcaaaaaagcggttagctccttcggtcctccgatcgttgtcagaagtaagttggccgcagtgttatcactcatggttatggcagcactgcataattctcttactgtcatgccatccgtaagatgcttttctgtgactggtgagtactcaaccaagtcattctgagaatagtgtatgcggcgaccgagttgctcttgcccggcgtcaatacgggataataccgcgccacatagcagaactttaaaagtgctcatcattggaaaacgttcttcggggcgaaaactctcaaggatcttaccgctgttgagatccagttcgatgtaacccactcgtgcacccaactgatcttcagcatcttttactttcaccagcgtttctgggtgagcaaaaacaggaaggcaaaatgccgcaaaaaagggaataagggcgacacggaaatgttgaatactcatactcttcctttttcaatattattgaagcatttatcagggttattgtctcatgagcggatacatatttgaatgtatttagaaaaataaacaaataggggttccgcgcacatttccccgaaaagtgccacctgacgtctaagaaaccattattatcatgacattaacctataaaaataggcgtatcacgaggccctttcgtc

SEQ ID NO: 8 - DNA, 4251 bp, Artificial sequence
  Synthetic
tcgcgcgtttcggtgatgacggtgaaaacctctgacacatgcagctcccggagacggtcacagcttgtctgtaagcggatgccgggagcagacaagcccgtcagggcgcgtcagcgggtgttggcgggtgtcggggctggcttaactatgcggcatcagagcagattgtactgagagtgcaccatatgcggtgtgaaataccgcacagatgcgtaaggagaaaataccgcatcaggcgccattcgccattcaggctgcgcaactgttgggaagggcgatcggtgcgggcctcttcgctattacgccagctggcgaaagggggatgtgctgcaaggcgattaagttgggtaacgccagggttttcccagtcacgacgttgtaaaacgacggccagtgaattctaatacgactcactatagggtaatacaagcttgcttgttctttttgcagaagctcagaataaacgctcaactttggcagatctgccaccatgcccctcaacgttagcttcaccaacaggaactatgacctcgactacgactcggtgcagccgtatttctactgcgacgaggaggagaacttctaccagcagcagcagcagagcgagctgcagcccccggcgcccagcgaggatatctggaagaaattcgagctgctgcccgcgccgcccctgtcccctagccgccgctccgggctctgctcgccctcctacgttgcggtcacacccttctcccttcggggagacaacgacggcggtggcgggagcttctccacggccgaccagctggagatggtgaccgagctgctgggaggagacatggtgaaccagagtttcatctgcgacccggacgacgagaccttcatcaaaaacatcatcatccaggactgtatgtggagcggcttctcggccgccgccaagctcgtctcagagaagctggcctcctaccaggctgcgcgcaaagacagcggcagcccgaaccccgcccgcggccacagcgtctgctccacctccagcttgtacctgcaggatctgagcgccgccgcctcagagtgcatcgacccctcggtggtcttcccctaccctctcaacgacagcagctcgcccaagtcctgcgcctcgcaagactccagcgccttctctccgtcctcggattctctgctctcctcgacggagtcctccccgcagggcagccccgagcccctggtgctccatgaggagacaccgcccaccaccagcagcgactctgaggaggaacaagaagatgaggaagaaatcgatgttgtttctgtggaaaagaggcaggctcctggcaaaaggtcagagtctggatcaccttctgctggaggccacagcaaacctcctcacagcccactggtcctcaagaggtgccacgtctccacacatcagcacaactacgcagcgcctccctccactcggaaggactatcctgctgccaagagggtcaagttggacagtgtcagagtcctgagacagatcagcaacaaccgaaaatgcaccagccccaggtcctcggacaccgaggagaatgtcaagaggcgaacacacaacgtcttggagcgccagaggaggaacgagctaaaacggagcttttttgccctgcgtgaccagatcccggagttggaaaacaatgaaaaggcccccaaggtagttatccttaaaaaagccacagcatacatcctgtccgtccaagcagaggagcaaaagctcatttctgaagaggacttgttgcggaaacgacgagaacagttgaaacacaaacttgaacagctacggaactcttgtgcgtaaggatcatcactagtgactgactaggatctggttaccactaaaccagcctcaagaacacccgaatggagtctctaagctacataataccaacttacactttacaaaatgttgtcccccaaaatgtagccattcgtatctgctcctaataaaaagaaagtttcttcacattctggatcctctagagtcgacctgcaggcatgcaagcttggcgtaatcatggtcatagctgtttcctgtgtgaaattgttatccgctcacaattccacacaacatacgagccggaagcataaagtgtaaagcctggggtgcctaatgagtgagctaactcacattaattgcgttgcgctcactgcccgctttccagtcgggaaacctgtcgtgccagctgcattaatgaatcggccaacgcgcggggagaggcggtttgcgtattgggcgctcttccgcttcctcgctcactgactcgctgcgctcggtcgttcggctgcggcgagcggtatcagctcactcaaaggcggtaatacggttatccacagaatcaggggataacgcaggaaagaacatgtgagcaaaaggccagcaaaaggccaggaaccgtaaaaaggccgcgttgctggcgtttttccataggctccgcccccctgacgagcatcacaaaaatcgacgctcaagtcagaggtggcgaaacccgacaggactataaagataccaggcgtttccccctggaagctccctcgtgcgctctcctgttccgaccctgccgcttaccggatacctgtccgcctttctcccttcgggaagcgtggcgctttctcatagctcacgctgtaggtatctcagttcggtgtaggtcgttcgctccaagctgggctgtgtgcacgaaccccccgttcagcccgaccgctgcgccttatccggtaactatcgtcttgagtccaacccggtaagacacgacttatcgccactggcagcagccactggtaacaggattagcagagcgaggtatgtaggcggtgctacagagttcttgaagtggtggcctaactacggctacactagaagaacagtatttggtatctgcgctctgctgaagccagttaccttcggaaaaagagttggtagctcttgatccggcaaacaaaccaccgctggtagcggtggtttttttgtttgcaagcagcagattacgcgcagaaaaaaaggatctcaagaagatcctttgatcttttctacggggtctgacgctcagtggaacgaaaactcacgttaagggattttggtcatgagattatcaaaaaggatcttcacctagatccttttaaattaaaaatgaagttttaaatcaatctaaagtatatatgagtaaacttggtctgacagttaccaatgcttaatcagtgaggcacctatctcagcgatctgtctatttcgttcatccatagttgcctgactccccgtcgtgtagataactacgatacgggagggcttaccatctggccccagtgctgcaatgataccgcgagacccacgctcaccggctccagatttatcagcaataaaccagccagccggaagggccgagcgcagaagtggtcctgcaactttatccgcctccatccagtctattaattgttgccgggaagctagagtaagtagttcgccagttaatagtttgcgcaacgttgttgccattgctacaggcatcgtggtgtcacgctcgtcgtttggtatggcttcattcagctccggttcccaacgatcaaggcgagttacatgatcccccatgttgtgcaaaaaagcggttagctccttcggtcctccgatcgttgtcagaagtaagttggccgcagtgttatcactcatggttatggcagcactgcataattctcttactgtcatgccatccgtaagatgcttttctgtgactggtgagtactcaaccaagtcattctgagaatagtgtatgcggcgaccgagttgctcttgcccggcgtcaatacgggataataccgcgccacatagcagaactttaaaagtgctcatcattggaaaacgttcttcggggcgaaaactctcaaggatcttaccgctgttgagatccagttcgatgtaacccactcgtgcacccaactgatcttcagcatcttttactttcaccagcgtttctgggtgagcaaaaacaggaaggcaaaatgccgcaaaaaagggaataagggcgacacggaaatgttgaatactcatactcttcctttttcaatattattgaagcatttatcagggttattgtctcatgagcggatacatatttgaatgtatttagaaaaataaacaaataggggttccgcgcacatttccccgaaaagtgccacctgacgtctaagaaaccattattatcatgacattaacctataaaaataggcgtatcacgaggccctttcgtc

SEQ ID NO: 9 - DNA, 4251 bp, Artificial sequence
  Synthetic
tcgcgcgtttcggtgatgacggtgaaaacctctgacacatgcagctcccggagacggtcacagcttgtctgtaagcggatgccgggagcagacaagcccgtcagggcgcgtcagcgggtgttggcgggtgtcggggctggcttaactatgcggcatcagagcagattgtactgagagtgcaccatatgcggtgtgaaataccgcacagatgcgtaaggagaaaataccgcatcaggcgccattcgccattcaggctgcgcaactgttgggaagggcgatcggtgcgggcctcttcgctattacgccagctggcgaaagggggatgtgctgcaaggcgattaagttgggtaacgccagggttttcccagtcacgacgttgtaaaacgacggccagtgaattctaatacgactcactatagggtaatacaagcttgcttgttctttttgcagaagctcagaataaacgctcaactttggcagatctgccaccatgcccctcaacgttagcttcaccaacaggaactatgacctcgactacgactcggtgcagccgtatttctactgcgacgaggaggagaacttctaccagcagcagcagcagagcgagctgcagcccccggcgcccagcgaggatatctggaagaaattcgagctgctgcccaccccgcccctgtcccctagccgccgctccgggctctgctcgccctcctacgttgcggtcacacccttctcccttcggggagacaacgacggcggtggcgggagcttctccacggccgaccagctggagatggtgaccgagctgctgggaggagacatggtgaaccagagtttcatctgcgacccggacgacgagaccttcatcaaaaacatcatcatccaggactgtatgtggagcggcttctcggccgccgccaagctcgtctcagagaagctggcctcctaccaggctgcgcgcaaagacagcggcagcccgaaccccgcccgcggccacagcgtctgctccacctccagcttgtacctgcaggatctgagcgccgccgcctcagagtgcatcgacccctcggtggtcttcccctaccctctcaacgacagcagctcgcccaagtcctgcgcctcgcaagactccagcgccttctctccgtcctcggattctctgctctcctcgacggagtcctccccgcagggcagccccgagcccctggtgctccatgaggagacaccgcccaccaccagcagcgactctgaggaggaacaagaagatgaggaagaaatcgatgttgtttctgtggaaaagaggcaggctcctggcaaaaggtcagagtctggatcaccttctgctggaggccacagcaaacctcctcacagcccactggtcctcaagaggtgccacgtctccacacatcagcacaactacgcagcgcctccctccactcggaaggactatcctgctgccaagagggtcaagttggacagtgtcagagtcctgagacagatcagcaacaaccgaaaatgcaccagccccaggtcctcggacaccgaggagaatgtcaagaggcgaacacacaacgtcttggagcgccagaggaggaacgagctaaaacggagcttttttgccctgcgtgaccagatcccggagttggaaaacaatgaaaaggcccccaaggtagttatccttaaaaaagccacagcatacatcctgtccgtccaagcagaggagcaaaagctcatttctgaagaggacttgttgcggaaacgacgagaacagttgaaacacaaacttgaacagctacggaactcttgtgcgtaaggatcatcactagtgactgactaggatctggttaccactaaaccagcctcaagaacacccgaatggagtctctaagctacataataccaacttacactttacaaaatgttgtcccccaaaatgtagccattcgtatctgctcctaataaaaagaaagtttcttcacattctggatcctctagagtcgacctgcaggcatgcaagcttggcgtaatcatggtcatagctgtttcctgtgtgaaattgttatccgctcacaattccacacaacatacgagccggaagcataaagtgtaaagcctggggtgcctaatgagtgagctaactcacattaattgcgttgcgctcactgcccgctttccagtcgggaaacctgtcgtgccagctgcattaatgaatcggccaacgcgcggggagaggcggtttgcgtattgggcgctcttccgcttcctcgctcactgactcgctgcgctcggtcgttcggctgcggcgagcggtatcagctcactcaaaggcggtaatacggttatccacagaatcaggggataacgcaggaaagaacatgtgagcaaaaggccagcaaaaggccaggaaccgtaaaaaggccgcgttgctggcgtttttccataggctccgcccccctgacgagcatcacaaaaatcgacgctcaagtcagaggtggcgaaacccgacaggactataaagataccaggcgtttccccctggaagctccctcgtgcgctctcctgttccgaccctgccgcttaccggatacctgtccgcctttctcccttcgggaagcgtggcgctttctcatagctcacgctgtaggtatctcagttcggtgtaggtcgttcgctccaagctgggctgtgtgcacgaaccccccgttcagcccgaccgctgcgccttatccggtaactatcgtcttgagtccaacccggtaagacacgacttatcgccactggcagcagccactggtaacaggattagcagagcgaggtatgtaggcggtgctacagagttcttgaagtggtggcctaactacggctacactagaagaacagtatttggtatctgcgctctgctgaagccagttaccttcggaaaaagagttggtagctcttgatccggcaaacaaaccaccgctggtagcggtggtttttttgtttgcaagcagcagattacgcgcagaaaaaaaggatctcaagaagatcctttgatcttttctacggggtctgacgctcagtggaacgaaaactcacgttaagggattttggtcatgagattatcaaaaaggatcttcacctagatccttttaaattaaaaatgaagttttaaatcaatctaaagtatatatgagtaaacttggtctgacagttaccaatgcttaatcagtgaggcacctatctcagcgatctgtctatttcgttcatccatagttgcctgactccccgtcgtgtagataactacgatacgggagggcttaccatctggccccagtgctgcaatgataccgcgagacccacgctcaccggctccagatttatcagcaataaaccagccagccggaagggccgagcgcagaagtggtcctgcaactttatccgcctccatccagtctattaattgttgccgggaagctagagtaagtagttcgccagttaatagtttgcgcaacgttgttgccattgctacaggcatcgtggtgtcacgctcgtcgtttggtatggcttcattcagctccggttcccaacgatcaaggcgagttacatgatcccccatgttgtgcaaaaaagcggttagctccttcggtcctccgatcgttgtcagaagtaagttggccgcagtgttatcactcatggttatggcagcactgcataattctcttactgtcatgccatccgtaagatgcttttctgtgactggtgagtactcaaccaagtcattctgagaatagtgtatgcggcgaccgagttgctcttgcccggcgtcaatacgggataataccgcgccacatagcagaactttaaaagtgctcatcattggaaaacgttcttcggggcgaaaactctcaaggatcttaccgctgttgagatccagttcgatgtaacccactcgtgcacccaactgatcttcagcatcttttactttcaccagcgtttctgggtgagcaaaaacaggaaggcaaaatgccgcaaaaaagggaataagggcgacacggaaatgttgaatactcatactcttcctttttcaatattattgaagcatttatcagggttattgtctcatgagcggatacatatttgaatgtatttagaaaaataaacaaataggggttccgcgcacatttccccgaaaagtgccacctgacgtctaagaaaccattattatcatgacattaacctataaaaataggcgtatcacgaggccctttcgtc

SEQ ID NO: 10 - DNA, 4018 bp, Artificial sequence
  Synthetic
tcgcgcgtttcggtgatgacggtgaaaacctctgacacatgcagctcccggagacggtcacagcttgtctgtaagcggatgccgggagcagacaagcccgtcagggcgcgtcagcgggtgttggcgggtgtcggggctggcttaactatgcggcatcagagcagattgtactgagagtgcaccatatgcggtgtgaaataccgcacagatgcgtaaggagaaaataccgcatcaggcgccattcgccattcaggctgcgcaactgttgggaagggcgatcggtgcgggcctcttcgctattacgccagctggcgaaagggggatgtgctgcaaggcgattaagttgggtaacgccagggttttcccagtcacgacgttgtaaaacgacggccagtgaattctaatacgactcactatagggtaatacaagcttgcttgttctttttgcagaagctcagaataaacgctcaactttggcagatctgccaccatggactacgactcgtaccagcactatttctacgactatgactgcggggaggatttctaccgctccacggcgcccagcgaggacatctggaagaaattcgagctggtgccatcgccccccacgtcgccgccctggggcttgggtcccggcgcaggggacccggcccccgggattggtcccccggagccgtggcccggagggtgcaccggagacgaagcggaatcccggggccactcgaaaggctggggcaggaactacgcctccatcatacgccgtgactgcatgtggagcggcttctcggcccgggaacggctggagagagctgtgagcgaccggctcgctcctggcgcgccccgggggaacccgcccaaggcgtccgccgccccggactgcactcccagcctcgaagccggcaacccggcgcccgccgccccctgtccgctgggcgaacccaagacccaggcctgctccgggtccgagagcccaagcgactcggagaatgaagaaattgatgttgtgacagtagagaagaggcagtctctgggtattcggaagccggtcaccatcacggtgcgagcagaccccctggatccctgcatgaagcatttccacatctccatccatcagcaacagcacaactatgctgcccgttttcctccagaaagctgctcccaagaagaggcttcagagaggggtccccaagaagaggttctggagagagatgctgcaggggaaaaggaagatgaggaggatgaagagattgtgagtcccccacctgtagaaagtgaggctgcccagtcctgccaccccaaacctgtcagttctgatactgaggatgtgaccaagaggaagaatcacaacttcctggagcgcaagaggcggaatgacctgcgttcgcgattcttggcgctgagggaccaggtgcccaccctggccagctgctccaaggcccccaaagtagtgatcctaagcaaggccttggaatacttgcaagccctggtgggggctgagaagaggatggctacagagaaaagacagctccgatgccggcagcagcagttgcagaaaagaattgcatacctcactggctactaaactagtgactgactaggatctggttaccactaaaccagcctcaagaacacccgaatggagtctctaagctacataataccaacttacactttacaaaatgttgtcccccaaaatgtagccattcgtatctgctcctaataaaaagaaagtttcttcacattctggatcctctagagtcgacctgcaggcatgcaagcttggcgtaatcatggtcatagctgtttcctgtgtgaaattgttatccgctcacaattccacacaacatacgagccggaagcataaagtgtaaagcctggggtgcctaatgagtgagctaactcacattaattgcgttgcgctcactgcccgctttccagtcgggaaacctgtcgtgccagctgcattaatgaatcggccaacgcgcggggagaggcggtttgcgtattgggcgctcttccgcttcctcgctcactgactcgctgcgctcggtcgttcggctgcggcgagcggtatcagctcactcaaaggcggtaatacggttatccacagaatcaggggataacgcaggaaagaacatgtgagcaaaaggccagcaaaaggccaggaaccgtaaaaaggccgcgttgctggcgtttttccataggctccgcccccctgacgagcatcacaaaaatcgacgctcaagtcagaggtggcgaaacccgacaggactataaagataccaggcgtttccccctggaagctccctcgtgcgctctcctgttccgaccctgccgcttaccggatacctgtccgcctttctcccttcgggaagcgtggcgctttctcatagctcacgctgtaggtatctcagttcggtgtaggtcgttcgctccaagctgggctgtgtgcacgaaccccccgttcagcccgaccgctgcgccttatccggtaactatcgtcttgagtccaacccggtaagacacgacttatcgccactggcagcagccactggtaacaggattagcagagcgaggtatgtaggcggtgctacagagttcttgaagtggtggcctaactacggctacactagaagaacagtatttggtatctgcgctctgctgaagccagttaccttcggaaaaagagttggtagctcttgatccggcaaacaaaccaccgctggtagcggtggtttttttgtttgcaagcagcagattacgcgcagaaaaaaaggatctcaagaagatcctttgatcttttctacggggtctgacgctcagtggaacgaaaactcacgttaagggattttggtcatgagattatcaaaaaggatcttcacctagatccttttaaattaaaaatgaagttttaaatcaatctaaagtatatatgagtaaacttggtctgacagttaccaatgcttaatcagtgaggcacctatctcagcgatctgtctatttcgttcatccatagttgcctgactccccgtcgtgtagataactacgatacgggagggcttaccatctggccccagtgctgcaatgataccgcgagacccacgctcaccggctccagatttatcagcaataaaccagccagccggaagggccgagcgcagaagtggtcctgcaactttatccgcctccatccagtctattaattgttgccgggaagctagagtaagtagttcgccagttaatagtttgcgcaacgttgttgccattgctacaggcatcgtggtgtcacgctcgtcgtttggtatggcttcattcagctccggttcccaacgatcaaggcgagttacatgatcccccatgttgtgcaaaaaagcggttagctccttcggtcctccgatcgttgtcagaagtaagttggccgcagtgttatcactcatggttatggcagcactgcataattctcttactgtcatgccatccgtaagatgcttttctgtgactggtgagtactcaaccaagtcattctgagaatagtgtatgcggcgaccgagttgctcttgcccggcgtcaatacgggataataccgcgccacatagcagaactttaaaagtgctcatcattggaaaacgttcttcggggcgaaaactctcaaggatcttaccgctgttgagatccagttcgatgtaacccactcgtgcacccaactgatcttcagcatcttttactttcaccagcgtttctgggtgagcaaaaacaggaaggcaaaatgccgcaaaaaagggaataagggcgacacggaaatgttgaatactcatactcttcctttttcaatattattgaagcatttatcagggttattgtctcatgagcggatacatatttgaatgtatttagaaaaataaacaaataggggttccgcgcacatttccccgaaaagtgccacctgacgtctaagaaaccattattatcatgacattaacctataaaaataggcgtatcacgaggccctttcgtc

SEQ ID NO: 11 - RNA, 738 nt, Homo sapiens
auggaaagcucugccaagauggagagcggcggcgccggccagcagccccagccgcagccccagcagcccuuccugccgcccgcagccuguuucuuugccacggccgcagccgcggcggccgcagccgccgcagcggcagcgcagagcgcgcagcagcagcagcagcagcagcagcagcagcagcagcagcaggcgccgcagcugagaccggcggccgacggccagcccucagggggcggucacaagucagcgcccaagcaagucaagcgacagcgcucgucuucgcccgaacugaugcgcugcaaacgccggcucaacuucagcggcuuuggcuacagccugccgcagcagcagccggccgccguggcgcgccgcaacgagcgcgagcgcaaccgcgucaaguuggucaaccugggcuuugccacccuucgggagcacguccccaacggcgcggccaacaagaagaugaguaagguggagacacugcgcucggcggucgaguacauccgcgcgcugcagcagcugcuggacgagcaugacgcggugagcgccgccuuccaggcaggcguccugucgcccaccaucucccccaacuacuccaacgacuugaacuccauggccggcucgccggucucauccuacucgucggacgagggcucuuacgacccgcucagccccgaggagcaggagcuucucgacuucaccaacugguucagaucugauaucacuagugacuga

SEQ ID NO: 12 - RNA, 3576 nt, Homo sapiens
auggagguggacaccgaggagaagcggcaucgcacgcgguccaaagggguucgaguucccguggaaccagccauacaagagcuguucagcugucccaccccuggcugugacggcaguggucaugucaguggcaaauaugcaagacacagaaguguauaugguugucccuuggcgaaaaaaagaaaaacacaagauaaacagccccaggaaccugcuccuaaacgaaagccauuugccgugaaagcagacagcuccucaguggaugagugugacgacagugaugggacugaggacauggaugagaaggaggaggaugagggggaggaguacuccgaggacaaugacgagccaggggaugaggacgaggaggacgaggagggggaccgggaggaggaggaggagaucgaggaggaggaugaggacgaugacgaggauggagaagauguggaggaugaagaagaggaagaggaggaggaggaggaggaggaagaggaagaagaaaacgaagaccaucaaaugaauugucacaauacucgaauaaugcaagacacagaaaaggaugauaacaauaaugacgaauaugacaauuacgaugaacugguggccaagucauuguuaaaccucggcaaaaucgcugaggaugcagccuaccgggccaggacugagucagaaaugaacagcaauaccuccaauagucuggaagacgauagugacaaaaacgaaaaccugggucggaaaagugaguugaguuuagacuuagacagugauguuguuagagaaacaguggacucccuuaaacuauuagcccaaggacacgguguugugcucucagaaaacaugaaugacagaaauuaugcagacagcaugucgcagcaagacaguagaaauaugaauuacgucauguuggggaagcccaugaacaauggacucauggaaaagaugguggaggagagcgaugaggaggugugucugagcagucuggaguguuugaggaaucagugcuucgaccuggccaggaagcucagugagaccaacccgcaggagaggaauccgcagcagaacaugaacauccgucagcauguccggccagaagaggacuucccaggaaggacgccggacagaaacuacucggacaugcugaaccucaugcggcuggaggagcaguugagcccccggucgagaguguuugccagcugugcgaaggaggaugggugucaugagcgggacgacgauaccaccucugugaacucggacaggucugaagagguguucgacaugaccaaggggaaccugacccugcuggagaaagccaucgcuuuggaaacggaaagagcaaaggccaugagggagaagauggccauggaagcugggaggagggacaauaugaggucauaugaggaccagucuccgagacaacuucccggggaggacagaaagccuaaauccagugacagccaugucaaaaagccauacuaugaucccucaagaacagaaaagaaagagagcaaguguccaacccccgggugugauggaaccggccacguaacugggcuguacccacaucaccgcagccuguccggaugcccgcacaaagauagggucccuccagaaauccuugccaugcaugaaaguguccucaagugccccacuccgggcugcacggggcgcgggcaugucaacagcaacaggaacucccaccgaagccucuccggaugcccgaucgcugcagcagagaaacuggccaaggcacaggaaaagcaccagagcugcgacguguccaaguccagccaggccucggaccgcgugcucaggccaaugugcuuugugaagcagcuggagauuccucaguauggcuacagaaacaauguccccacaacuacgccgcguuccaaccuggccaaggagcucgagaaauauuccaagaccucguuugaauacaacaguuacgacaaccauacuuauggcaagcgagccauagcucccaaggugcaaaccagggauauaucccccaaaggauaugaugaugcgaagcgguacugcaaggaccccagccccagcagcagcagcaccagcagcuacgcgcccagcagcagcagcaaccugagcugcggcgggggcagcagcgccagcagcacgugcagcaagagcagcuucgacuacacgcacgacauggaggcggcccacauggcggccaccgccauccucaaccuguccacgcgcugccgcgagaugccgcagaaccugagcaccaagccgcaggaccugugcgccacgcggaacccugacauggagguggaugagaacgggacccuggaccucagcaugaacaagcagaggccgcgggacagcugcugccccauccugaccccucuggagcccauguccccccagcagcaggcagugaugaacaaccgguguuuccagcugggcgagggcgacugcugggacuugcccguagacuacaccaaaaugaaaccccggaggauagacgaggacgaguccaaagacauuacuccagaagacuuggacccauuccaggaggcucuagaagaaagacgguaucccggggaggugaccaucccaagucccaaacccaaguacccucagugcaaggagagcaaaaaggacuuaauaacucugucuggcugcccccuggcggacaaaagcauucgaaguaugcuggccaccagcucccaagaacucaagugccccacgccuggcugugaugguucuggacauaucaccggcaauuaugcuucucaucggagccuuucagguugcccaagagcaaagaaaagugguaucaggauagcacagagcaaagaagauaaagaagaucaagaacccaucagguguccgguccccgggugcgacggccagggccacaucacugggaaguacgcgucccaucgcagcgccuccgggugccccuuggcggccaagaggcagaaagacggguaccugaauggcucccaguucuccuggaagucggucaagacggaaggcauguccugccccacgccaggaugcgacggcucaggccacgucagcggcagcuuccucacacaccgcagcuugucaggaugcccgagagccacgucagcgaugaagaaggcaaagcuuucuggagagcagaugcugaccaucaaacagcgggccagcaacgguauagaaaaugaugaagaaaucaaacaguuagaugaagaaaucaaggagcuaaaugaauccaauucccagauggaagccgauaugauuaaacucagaacucagauuaccacgauggagagcaaccugaagaccaucgaagaggagaacaaagugauugagcagcagaacgagucucuccuccacgagcuggcgaaccugagccagucucugauccacagccuggcuaacauccagcugccgcacauggauccaaucaaugaacaaaauuuugaugcuuacgugacuacuuugacggaaauguauacaaaucaagaucguuaucagaguccagaaaauaaagcccuacuggaaaauauaaagcaggcugugagaggaauucaggucagaucugauaucacuagugacuga

SEQ ID NO: 13 - RNA, 1281 nt, Homo sapiens
augggcgagccucagccccaagguccuccaagcuggacagacgagugucucaguucucaggacgaggagcacgaggcagacaagaaggaggacgaccucgaagccaugaacgcagaggaggacucacugaggaacgggggagaggaggaggacgaagaugaggaccuggaagaggaggaagaagaggaagaggaggaugacgaucaaaagcccaagagacgcggccccaaaaagaagaagaugacuaaggcucgccuggagcguuuuaaauugagacgcaugaaggcuaacgcccgggagcggaaccgcaugcacggacugaacgcggcgcuagacaaccugcgcaagguggugccuugcuauucuaagacgcagaagcuguccaaaaucgagacucugcgcuuggccaagaacuacaucugggcucugucggagauccugcgcucaggcaaaagcccagaccuggucuccuucguucagacgcuuugcaagggcuuaucccaacccaccaccaaccugguugcgggcugccugcaacucaauccucggacuuuucugccugagcagaaccaggacaugcccccccaccugccgacggccagcgcuuccuucccuguacaccccuacuccuaccagucgccugggcugcccaguccgccuuacgguaccauggacagcucccaugucuuccacguuaagccuccgccgcacgccuacagcgcagcgcuggagcccuucuuugaaagcccucugacugauugcaccagcccuuccuuugauggaccccucagcccgccgcucagcaucaauggcaacuucucuuucaaacacgaaccguccgccgaguuugagaaaaauuaugccuuuaccaugcacuauccugcagcgacacuggcaggggcccaaagccacggaucaaucuucucaggcaccgcugccccucgcugcgagauccccauagacaauauuauguccuucgauagccauucacaucaugagcgagucaugagugcccagcucaaugccauauuucaugauuagaggcacgccaguuucaccauuuccgggaaacgaacccacugugcuuacagugacugucguguuuacaaaaggcagcccuuuggguacuacugcugcaaagugcaaauacuccaagcuucaagugauauauguauuuauugucauuacugccuuuggaagaaacaggggaucaaaguuccuguucaccuuauguauuauuuucuauagcucuucuauuuaaaaaauaaaaaaauacaguaa

SEQ ID NO: 14 - RNA, 1311 nt, Artificial sequence
  Synthetic
auggcgaccgcagcgucuaaccacuacagccugcucaccuccagcgccuccaucgugcacgccgagccgcccggcggcaugcagcagggcgcggggggcuaccgcgaagcgcagagccuggugcagggcgacuacggcgcucugcagagcaacggacacccgcucagccacgcucaccaguggaucacagcgcugucccacggcggcggcgggggcggcggcgacggcuccccgugguccaccagcccccugggccagccggacaucaagcccucggugguggugcagcagggcggccgcggagacgagcugcacgggccaggcgcccugcagcagcagcaucagcagcagcaacagcaacagcagcagcaacagcagcaacagcagcagcagcagcagcaacagcggccgccgcaucuggugcaccacgccgcuaaccaccacccgggacccggggcauggcggagcgcggcggcugcagcgcaccucccacccuccaugggagcguccaacggcggcuugcucuacucgcagcccagcuucacggugaacggcaugcugggcgccggcgggcagucggccgggcugcaccaccacggccugcgggacgcgcacgacgagccacaccaugccgaccaccacccgcacccgcacucgcacccacaccagcagccgccgcccccgccgcccccgcaggguccgccuggccacccaggcgcgcaccacgacccgcacucggacgaggacacgccgaccucggacgaccuggagcaguucgccaagcaguucaagcagcggcggaucaaacugggauuuacacaagcggacguggggcuggcucugggcacccuguauggcaacguguucucgcagaccaccaucugcagguuugaggcccugcagcugagcuucaagaacaugugcaagcugaagccuuuguugaacaagugguuggaggaggcggacucguccucgggcagccccacgagcauagacaagaucgcagcgcaagggcgcaagcggaaaaagcggaccuccaucgaggugagcgucaagggggcucuggagagccauuuccucaaaugccccaagcccucggcccaggagaucaccucccucgcggacagcuuacagcuggagaaggagguggugagaguuugguuuuguaacaggagacagaaagagaaaaggaugaccccucccggagggacucugccgggcgccgaggauguguacggggggaguagggacacuccaccacaccacggggugcagacgcccguccagagaucaucacuagugacugacuag

SEQ ID NO: 15 - RNA, 1332 nt, Homo sapiens
auggcgaccgcagcgucuaaccacuacagccugcucaccuccagcgccuccaucgugcacgccgagccgcccggcggcaugcagcagggcgcggggggcuaccgcgaagcgcagagccuggugcagggcgacuacggcgcucugcagagcaacggacacccgcucagccacgcucaccaguggaucaccgcgcugucccacggcggcggcggcgggggcgguggcggcggcggggggggcgggggcggcggcgggggcggcggcgacggcuccccgugguccaccagcccccugggccagccggacaucaagcccucggugguggugcagcagggcggccgcggagacgagcugcacgggccaggcgcccugcagcagcagcaucagcagcagcaacagcaacagcagcagcaacagcagcaacagcagcagcagcagcagcaacagcggccgccgcaucuggugcaccacgccgcuaaccaccacccgggacccggggcauggcggagcgcggcggcugcagcgcaccucccacccuccaugggagcguccaacggcggcuugcucuacucgcagcccagcuucacggugaacggcaugcugggcgccggcgggcagccggccggucugcaccaccacggccugcgggacgcgcacgacgagccacaccaugccgaccaccacccgcacccgcacucgcacccacaccagcagccgccgcccccgccgcccccgcaggguccgccuggccacccaggcgcgcaccacgacccgcacucggacgaggacacgccgaccucggacgaccuggagcaguucgccaagcaguucaagcagcggcggaucaaacugggauuuacccaagcggacguggggcuggcucugggcacccuguauggcaacguguucucgcagaccaccaucugcagguuugaggcccugcagcugagcuucaagaacaugugcaagcugaagccuuuguugaacaagugguuggaggaggcggacucguccucgggcagccccacgagcauagacaagaucgcagcgcaagggcgcaagcggaaaaagcggaccuccaucgaggugagcgucaagggggcucuggagagccauuuccucaaaugccccaagcccucggcccaggagaucaccucccucgcggacagcuuacagcuggagaaggagguggugagaguuugguuuuguaacaggagacagaaagagaaaaggaugaccccucccggagggacucugccgggcgccgaggauguguacggggggaguagggacacuccaccacaccacggggugcagacgcccguccaguga

SEQ ID NO: 16 - RNA, 1215 nt, Homo sapiens
ggguaauacaagcuugcuuguucuuuuugcagaagcucagaauaaacgcucaacuuuggcagaucugccaccauggagcuacugucgccaccgcuccgcgacguagaccugacggcccccgacggcucucucugcuccuuugccacaacggacgacuucuaugacgacccguguuucgacuccccggaccugcgcuucuucgaagaccuggacccgcgccugaugcacgugggcgcgcuccugaaacccgaagagcacucgcacuuccccgcggcggugcacccggccccgggcgcacgugaggacgagcaugugcgcgcgcccagcgggcaccaccaggcgggccgcugccuacugugggccugcaaggcgugcaagcgcaagaccaccaacgccgaccgccgcaaggccgccaccaugcgcgagcggcgccgccugagcaaaguaaaugaggccuuugagacacucaagcgcugcacgucgagcaauccaaaccagcgguugcccaagguggagauccugcgcaacgccauccgcuauaucgagggccugcaggcucugcugcgcgaccaggacgccgcgcccccuggcgccgcagccgccuucuaugcgccgggcccgcugcccccgggccgcggcggcgagcacuacagcggcgacuccgacgcguccagcccgcgcuccaacugcuccgacggcaugauggacuacagcggccccccgagcggcgcccggcggcggaacugcuacgaaggcgccuacuacaacgaggcgcccagcgaacccaggcccgggaagagugcggcggugucgagccuagacugccuguccagcaucguggagcgcaucuccaccgagagcccugcggcgcccgcccuccugcuggcggacgugccuucugagucgccuccgcgcaggcaagaggcugccgcccccagcgagggagagagcagcggcgaccccacccagucaccggacgccgccccgcagugcccugcgggugcgaaccccaacccgauauaccaggugcucugaacuagugacugacuaggaucugguuaccacuaaaccagccucaagaacacccgaauggagucucuaagcuacauaauaccaacuuacacuuuacaaaauguugucccccaaaauguagccauucguaucugcuccuaauaaaaagaaaguuucuucacauucuggauccucuagagucga